European Patent Specification EP 3 730 519 B1, published September 13, 2023. Title: B Cell Malignancy Recognizing Antibody or Antigen Binding Fragment Thereof, Chimeric Antigen Receptor Comprising The Same and Uses Thereof. Applicant: AbClon Inc. The sequence listing filed with the application follows.

SEQUENCE LISTING (200 sequences)

SEQ ID NO: 1 - protein, 5 aa, Artificial Sequence
  Amino acid sequence of CDRH1 of CD19_8.1 antibody
DYYMS

SEQ ID NO: 2 - protein, 17 aa, Artificial Sequence
  Amino acid sequence of CDRH2 of CD19_8.1 antibody
GIYYDDSSQYYADSVKG

SEQ ID NO: 3 - protein, 18 aa, Artificial Sequence
  Amino acid sequence of CDRH3 of CD19_8.1 antibody
GPLFCNDRTCSYYYAMDV

SEQ ID NO: 4 - protein, 13 aa, Artificial Sequence
  Amino acid sequence of CDRL1 of CD19_8.1 antibody
TGSSSNIGSNAVY

SEQ ID NO: 5 - protein, 7 aa, Artificial Sequence
  Amino acid sequence of CDRL2 of CD19_8.1 antibody
DDNHRPS

SEQ ID NO: 6 - protein, 11 aa, Artificial Sequence
  Amino acid sequence of CDRL3 of CD19_8.1 antibody
GTWDYSLSGYV

SEQ ID NO: 7 - protein, 17 aa, Artificial Sequence
  Amino acid sequence of CDRH2 of affinity matured clone 2B1
GIYYDGSARYYADSVKG

SEQ ID NO: 8 - protein, 17 aa, Artificial Sequence
  Amino acid sequence of CDRH2 of affinity matured clone B12
GIYYDGSAKYYADSVKG

SEQ ID NO: 9 - protein, 17 aa, Artificial Sequence
  Amino acid sequence of CDRH2 of affinity matured clone T2H3
GIYYDGSAKYYADSVKG

SEQ ID NO: 10 - protein, 17 aa, Artificial Sequence
  Amino acid sequence of CDRH2 of affinity matured clone T3C1
GIYYDGSASYYADSVKG

SEQ ID NO: 11 - protein, 17 aa, Artificial Sequence
  Amino acid sequence of CDRH2 of affinity matured clone D10
GIYYDGSAVYYADSVKG

SEQ ID NO: 12 - protein, 17 aa, Artificial Sequence
  Amino acid sequence of CDRH2 of affinity matured clone F6
GIYYDGSAKYYADSVKG

SEQ ID NO: 13 - protein, 17 aa, Artificial Sequence
  Amino acid sequence of CDRH2 of affinity matured clone B2
GIYYDGSTKYYADSVKG

SEQ ID NO: 14 - protein, 17 aa, Artificial Sequence
  Amino acid sequence of CDRH2 of affinity matured clone B6
GIYYDGSTAYYADSVKG

SEQ ID NO: 15 - protein, 17 aa, Artificial Sequence
  Amino acid sequence of CDRH2 of affinity matured clone 2F1
GIYYDGSSQGWSSSVKG

SEQ ID NO: 16 - protein, 17 aa, Artificial Sequence
  Amino acid sequence of CDRH2 of affinity matured clone C8
GIYYDGSQLYYADSVKG

SEQ ID NO: 17 - protein, 17 aa, Artificial Sequence
  Amino acid sequence of CDRH2 of affinity matured clone D4
GIYYDGSSQSMAGSVKG

SEQ ID NO: 18 - protein, 17 aa, Artificial Sequence
  Amino acid sequence of CDRH2 of affinity matured clone B5
GIYYDGSSQGMTNSVKG

SEQ ID NO: 19 - protein, 17 aa, Artificial Sequence
  Amino acid sequence of CDRH2 of affinity matured clone G4
GIYYDGSSQTLLPSVKG

SEQ ID NO: 20 - protein, 17 aa, Artificial Sequence
  Amino acid sequence of CDRH2 of affinity matured clone A7
GIYYDASWTYYADSVKG

SEQ ID NO: 21 - protein, 17 aa, Artificial Sequence
  Amino acid sequence of CDRH2 of affinity matured clone D12
GIYYDASTKYYADSVKG

SEQ ID NO: 22 - protein, 17 aa, Artificial Sequence
  Amino acid sequence of CDRH2 of affinity matured clone E2
GIYYDASIRYYADSVKG

SEQ ID NO: 23 - protein, 17 aa, Artificial Sequence
  Amino acid sequence of CDRH2 of affinity matured clone T2A1
GIYYDASVKYYADSVKG

SEQ ID NO: 24 - protein, 17 aa, Artificial Sequence
  Amino acid sequence of CDRH2 of affinity matured clone T3H9
GIYYDASAEYYADSVKG

SEQ ID NO: 25 - protein, 17 aa, Artificial Sequence
  Amino acid sequence of CDRH2 of affinity matured clone 2G1
GIYYDSSTRYYADSVKG

SEQ ID NO: 26 - protein, 17 aa, Artificial Sequence
  Amino acid sequence of CDRH2 of affinity matured clone C4
GIYYDSSMRYYADSVKG

SEQ ID NO: 27 - protein, 17 aa, Artificial Sequence
  Amino acid sequence of CDRH2 of affinity matured clone C5
GIYYDSSMRYYADSVKG

SEQ ID NO: 28 - protein, 17 aa, Artificial Sequence
  Amino acid sequence of CDRH2 of affinity matured clone D1
GIYYDSSAKYYADSVKG

SEQ ID NO: 29 - protein, 17 aa, Artificial Sequence
  Amino acid sequence of CDRH2 of affinity matured clone D2
GIYYDSSTDYYADSVKG

SEQ ID NO: 30 - protein, 17 aa, Artificial Sequence
  Amino acid sequence of CDRH2 of affinity matured clone E1
GIYYDSSVTYYADSVKG

SEQ ID NO: 31 - protein, 17 aa, Artificial Sequence
  Amino acid sequence of CDRH2 of affinity matured clone F3
GIYYDSSARYYADSVKG

SEQ ID NO: 32 - protein, 17 aa, Artificial Sequence
  Amino acid sequence of CDRH2 of affinity matured clone T2C1
GIYYDSSQDYYADSVKG

SEQ ID NO: 33 - protein, 17 aa, Artificial Sequence
  Amino acid sequence of CDRH2 of affinity matured clone T2H1
GIYYDSSQDYYADSVKG

SEQ ID NO: 34 - protein, 17 aa, Artificial Sequence
  Amino acid sequence of CDRH2 of affinity matured clone T2H5
GIYYDSSAKYYADSVKG

SEQ ID NO: 35 - protein, 17 aa, Artificial Sequence
  Amino acid sequence of CDRH2 of affinity matured clone T3B8
GIYYDSSVMYYADSVKG

SEQ ID NO: 36 - protein, 17 aa, Artificial Sequence
  Amino acid sequence of CDRH2 of affinity matured clone A12
GIYYDGTVLYYADSVKG

SEQ ID NO: 37 - protein, 17 aa, Artificial Sequence
  Amino acid sequence of CDRH2 of affinity matured clone C2
GIYYDGTNQYYADSVKG

SEQ ID NO: 38 - protein, 17 aa, Artificial Sequence
  Amino acid sequence of CDRH2 of affinity matured clone D7
GIYYDGTAFYYADSVKG

SEQ ID NO: 39 - protein, 17 aa, Artificial Sequence
  Amino acid sequence of CDRH2 of affinity matured clone E3
GIYYDGTAMYYADSVKG

SEQ ID NO: 40 - protein, 17 aa, Artificial Sequence
  Amino acid sequence of CDRH2 of affinity matured clone H10
GIYYDGTNVYYADSVKG

SEQ ID NO: 41 - protein, 17 aa, Artificial Sequence
  Amino acid sequence of CDRH2 of affinity matured clone T3F5
GIYYDGTAKYYADSVKG

SEQ ID NO: 42 - protein, 17 aa, Artificial Sequence
  Amino acid sequence of CDRH2 of affinity matured clone A10
GIYYDGIYRYYADSVKG

SEQ ID NO: 43 - protein, 17 aa, Artificial Sequence
  Amino acid sequence of CDRH2 of affinity matured clone T3H1
GIYYDGAVQYYADSVKG

SEQ ID NO: 44 - protein, 17 aa, Artificial Sequence
  Amino acid sequence of CDRH2 of affinity matured clone B1
GIYYDGDVRYYADSVKG

SEQ ID NO: 45 - protein, 17 aa, Artificial Sequence
  Amino acid sequence of CDRH2 of affinity matured clone B7
GIYYDGFAPYYADSVKG

SEQ ID NO: 46 - protein, 17 aa, Artificial Sequence
  Amino acid sequence of CDRH2 of affinity matured clone D8
GIYYDGLHQYYADSVKG

SEQ ID NO: 47 - protein, 17 aa, Artificial Sequence
  Amino acid sequence of CDRH2 of affinity matured clone E12
GIYYDSFVPYYADSVKG

SEQ ID NO: 48 - protein, 17 aa, Artificial Sequence
  Amino acid sequence of CDRH2 of affinity matured clone T2A12
GIYYDGHQQYYADSVKG

SEQ ID NO: 49 - protein, 13 aa, Artificial Sequence
  Amino acid sequence of CDRL1 of affinity matured clone 2B1
VGGVSNIGSNAVY

SEQ ID NO: 50 - protein, 13 aa, Artificial Sequence
  Amino acid sequence of CDRL1 of affinity matured clone B12
AGHYSNIGSNAVY

SEQ ID NO: 51 - protein, 13 aa, Artificial Sequence
  Amino acid sequence of CDRL1 of affinity matured clone T2H3
GGGISNIGSNAVY

SEQ ID NO: 52 - protein, 13 aa, Artificial Sequence
  Amino acid sequence of CDRL1 of affinity matured clone T3C1
SGGPSNIGSNAVY

SEQ ID NO: 53 - protein, 13 aa, Artificial Sequence
  Amino acid sequence of CDRL1 of affinity matured clone D10
WGDYSNIGSNAVY

SEQ ID NO: 54 - protein, 13 aa, Artificial Sequence
  Amino acid sequence of CDRL1 of affinity matured clone F6
WGLPSNIGSNAVY

SEQ ID NO: 55 - protein, 13 aa, Artificial Sequence
  Amino acid sequence of CDRL1 of affinity matured clone B2
AGGVSNIGSNAVY

SEQ ID NO: 56 - protein, 13 aa, Artificial Sequence
  Amino acid sequence of CDRL1 of affinity matured clone B6
NGTPSNIGSNAVY

SEQ ID NO: 57 - protein, 13 aa, Artificial Sequence
  Amino acid sequence of CDRL1 of affinity matured clone 2F1
YGQPSNIGSNAVY

SEQ ID NO: 58 - protein, 13 aa, Artificial Sequence
  Amino acid sequence of CDRL1 of affinity matured clone C8
KGGMSNIGSNAVY

SEQ ID NO: 59 - protein, 13 aa, Artificial Sequence
  Amino acid sequence of CDRL1 of affinity matured clone D4
TGGVSNIGSNAVY

SEQ ID NO: 60 - protein, 13 aa, Artificial Sequence
  Amino acid sequence of CDRL1 of affinity matured clone B5
HGTPSNIGSNAVY

SEQ ID NO: 61 - protein, 13 aa, Artificial Sequence
  Amino acid sequence of CDRL1 of affinity matured clone G4
VGKPSNIGSNAVY

SEQ ID NO: 62 - protein, 13 aa, Artificial Sequence
  Amino acid sequence of CDRL1 of affinity matured clone A7
TGNPSNIGSNAVY

SEQ ID NO: 63 - protein, 13 aa, Artificial Sequence
  Amino acid sequence of CDRL1 of affinity matured clone D12
RGSASNIGSNAVY

SEQ ID NO: 64 - protein, 13 aa, Artificial Sequence
  Amino acid sequence of CDRL1 of affinity matured clone E2
KGMISNIGSNAVY

SEQ ID NO: 65 - protein, 13 aa, Artificial Sequence
  Amino acid sequence of CDRL1 of affinity matured clone T2A1
AGKPSNIGSNAVY

SEQ ID NO: 66 - protein, 13 aa, Artificial Sequence
  Amino acid sequence of CDRL1 of affinity matured clone T3H9
SGMLSNIGSNAVY

SEQ ID NO: 67 - protein, 13 aa, Artificial Sequence
  Amino acid sequence of CDRL1 of affinity matured clone 2G1
KGSFSNIGSNAVY

SEQ ID NO: 68 - protein, 13 aa, Artificial Sequence
  Amino acid sequence of CDRL1 of affinity matured clone C4
GGQPSNIGSNAVY

SEQ ID NO: 69 - protein, 13 aa, Artificial Sequence
  Amino acid sequence of CDRL1 of affinity matured clone C5
KGGMSNIGSNAVY

SEQ ID NO: 70 - protein, 13 aa, Artificial Sequence
  Amino acid sequence of CDRL1 of affinity matured clone D1
SGGPSNIGSNAVY

SEQ ID NO: 71 - protein, 13 aa, Artificial Sequence
  Amino acid sequence of CDRL1 of affinity matured clone D2
QGQPSNIGSNAVY

SEQ ID NO: 72 - protein, 13 aa, Artificial Sequence
  Amino acid sequence of CDRL1 of affinity matured clone E1
TGNPSNIGSNAVY

SEQ ID NO: 73 - protein, 13 aa, Artificial Sequence
  Amino acid sequence of CDRL1 of affinity matured clone F3
TGSSSNIGSAPLY

SEQ ID NO: 74 - protein, 13 aa, Artificial Sequence
  Amino acid sequence of CDRL1 of affinity matured clone T2C1
RGGPSNIGSNAVY

SEQ ID NO: 75 - protein, 13 aa, Artificial Sequence
  Amino acid sequence of CDRL1 of affinity matured clone T2H1
QGGYSNIGSNAVY

SEQ ID NO: 76 - protein, 13 aa, Artificial Sequence
  Amino acid sequence of CDRL1 of affinity matured clone T2H5
SGNPSNIGSNAVY

SEQ ID NO: 77 - protein, 13 aa, Artificial Sequence
  Amino acid sequence of CDRL1 of affinity matured clone T3B8
EGSPSNIGSNAVY

SEQ ID NO: 78 - protein, 13 aa, Artificial Sequence
  Amino acid sequence of CDRL1 of affinity matured clone A12
QGGPSNIGSNAVY

SEQ ID NO: 79 - protein, 13 aa, Artificial Sequence
  Amino acid sequence of CDRL1 of affinity matured clone C2
TGGLSNIGSNAVY

SEQ ID NO: 80 - protein, 13 aa, Artificial Sequence
  Amino acid sequence of CDRL1 of affinity matured clone D7
EGQPSNIGSNAVY

SEQ ID NO: 81 - protein, 13 aa, Artificial Sequence
  Amino acid sequence of CDRL1 of affinity matured clone E3
SGGYSNIGSNAVY

SEQ ID NO: 82 - protein, 13 aa, Artificial Sequence
  Amino acid sequence of CDRL1 of affinity matured clone H10
LGGYSNIGSNAVY

SEQ ID NO: 83 - protein, 13 aa, Artificial Sequence
  Amino acid sequence of CDRL1 of affinity matured clone T3F5
HGQPSNIGSNAVY

SEQ ID NO: 84 - protein, 13 aa, Artificial Sequence
  Amino acid sequence of CDRL1 of affinity matured clone A10
SGDPSNIGSNAVY

SEQ ID NO: 85 - protein, 13 aa, Artificial Sequence
  Amino acid sequence of CDRL1 of affinity matured clone T3H1
DGGYSNIGSNAVY

SEQ ID NO: 86 - protein, 13 aa, Artificial Sequence
  Amino acid sequence of CDRL1 of affinity matured clone B1
VGSPSNIGSNAVY

SEQ ID NO: 87 - protein, 13 aa, Artificial Sequence
  Amino acid sequence of CDRL1 of affinity matured clone B7
RGTPSNIGSNAVY

SEQ ID NO: 88 - protein, 13 aa, Artificial Sequence
  Amino acid sequence of CDRL1 of affinity matured clone D8
VGNLSNIGSNAVY

SEQ ID NO: 89 - protein, 13 aa, Artificial Sequence
  Amino acid sequence of CDRL1 of affinity matured clone E12
AGSASNIGSNAVY

SEQ ID NO: 90 - protein, 13 aa, Artificial Sequence
  Amino acid sequence of CDRL1 of affinity matured clone T2A12
TGSSSNIGSAPTY

SEQ ID NO: 91 - protein, 127 aa, Artificial Sequence
  Amino acid sequence of heavy chain variable region of CD19_8.1 antibody
EVQLLESGGGLVQPGGSLRLSCAASGFTFSDYYMSWVRQAPGKGLEWVSGIYYDDSSQYYADSVKGRFTISRDNSKNTLYLQMNSLRAEDTAVYYCAKGPLFCNDRTCSYYYAMDVWGQGTLVTVSS

SEQ ID NO: 92 - protein, 127 aa, Artificial Sequence
  Amino acid sequence of heavy chain variable region of affinity matured clone 2B1
EVQLLESGGGLVQPGGSLRLSCAASGFTFSDYYMSWVRQAPGKGLEWVSGIYYDGSARYYADSVKGRFTISRDNSKNTLYLQMNSLRAEDTAVYYCAKGPLFCNDRTCSYYYAMDVWGQGTLVTVSS

SEQ ID NO: 93 - protein, 127 aa, Artificial Sequence
  Amino acid sequence of heavy chain variable region of affinity matured clone B12
EVQLLESGGGLVQPGGSLRLSCAASGFTFSDYYMSWVRQAPGKGLEWVSGIYYDGSAKYYADSVKGRFTISRDNSKNTLYLQMNSLRAEDTAVYYCAKGPLFCNDRTCSYYYAMDVWGQGTLVTVSS

SEQ ID NO: 94 - protein, 127 aa, Artificial Sequence; identical to SEQ ID NO: 93
  Amino acid sequence of heavy chain variable region of affinity matured clone T2H3

SEQ ID NO: 95 - protein, 127 aa, Artificial Sequence
  Amino acid sequence of heavy chain variable region of affinity matured clone T3C1
EVQLLESGGGLVQPGGSLRLSCAASGFTFSDYYMSWVRQAPGKGLEWVSGIYYDGSASYYADSVKGRFTISRDNSKNTLYLQMNSLRAEDTAVYYCAKGPLFCNDRTCSYYYAMDVWGQGTLVTVSS

SEQ ID NO: 96 - protein, 127 aa, Artificial Sequence
  Amino acid sequence of heavy chain variable region of affinity matured clone D10
EVQLLESGGGLVQPGGSLRLSCAASGFTFSDYYMSWVRQAPGKGLEWVSGIYYDGSAVYYADSVKGRFTISRDNSKNTLYLQMNSLRAEDTAVYYCAKGPLFCNDRTCSYYYAMDVWGQGTLVTVSS

SEQ ID NO: 97 - protein, 127 aa, Artificial Sequence; identical to SEQ ID NO: 93
  Amino acid sequence of heavy chain variable region of affinity matured clone F6

SEQ ID NO: 98 - protein, 127 aa, Artificial Sequence
  Amino acid sequence of heavy chain variable region of affinity matured clone B2
EVQLLESGGGLVQPGGSLRLSCAASGFTFSDYYMSWVRQAPGKGLEWVSGIYYDGSTKYYADSVKGRFTISRDNSKNTLYLQMNSLRAEDTAVYYCAKGPLFCNDRTCSYYYAMDVWGQGTLVTVSS

SEQ ID NO: 99 - protein, 127 aa, Artificial Sequence
  Amino acid sequence of heavy chain variable region of affinity matured clone B6
EVQLLESGGGLVQPGGSLRLSCAASGFTFSDYYMSWVRQAPGKGLEWVSGIYYDGSTAYYADSVKGRFTISRDNSKNTLYLQMNSLRAEDTAVYYCAKGPLFCNDRTCSYYYAMDVWGQGTLVTVSS

SEQ ID NO: 100 - protein, 127 aa, Artificial Sequence
  Amino acid sequence of heavy chain variable region of affinity matured clone 2F1
EVQLLESGGGLVQPGGSLRLSCAASGFTFSDYYMSWVRQAPGKGLEWVSGIYYDGSSQGWSSSVKGRFTISRDNSKNTLYLQMNSLRAEDTAVYYCAKGPLFCNDRTCSYYYAMDVWGQGTLVTVSS

SEQ ID NO: 101 - protein, 127 aa, Artificial Sequence
  Amino acid sequence of heavy chain variable region of affinity matured clone C8
EVQLLESGGGLVQPGGSLRLSCAASGFTFSDYYMSWVRQAPGKGLEWVSGIYYDGSQLYYADSVKGRFTISRDNSKNTLYLQMNSLRAEDTAVYYCAKGPLFCNDRTCSYYYAMDVWGQGTLVTVSS

SEQ ID NO: 102 - protein, 127 aa, Artificial Sequence
  Amino acid sequence of heavy chain variable region of affinity matured clone D4
EVQLLESGGGLVQPGGSLRLSCAASGFTFSDYYMSWVRQAPGKGLEWVSGIYYDGSSQSMAGSVKGRFTISRDNSKNTLYLQMNSLRAEDTAVYYCAKGPLFCNDRTCSYYYAMDVWGQGTLVTVSS

SEQ ID NO: 103 - protein, 127 aa, Artificial Sequence
  Amino acid sequence of heavy chain variable region of affinity matured clone B5
EVQLLESGGGLVQPGGSLRLSCAASGFTFSDYYMSWVRQAPGKGLEWVSGIYYDGSSQGMTNSVKGRFTISRDNSKNTLYLQMNSLRAEDTAVYYCAKGPLFCNDRTCSYYYAMDVWGQGTLVTVSS

SEQ ID NO: 104 - protein, 127 aa, Artificial Sequence
  Amino acid sequence of heavy chain variable region of affinity matured clone G4
EVQLLESGGGLVQPGGSLRLSCAASGFTFSDYYMSWVRQAPGKGLEWVSGIYYDGSSQTLLPSVKGRFTISRDNSKNTLYLQMNSLRAEDTAVYYCAKGPLFCNDRTCSYYYAMDVWGQGTLVTVSS

SEQ ID NO: 105 - protein, 127 aa, Artificial Sequence
  Amino acid sequence of heavy chain variable region of affinity matured clone A7
EVQLLESGGGLVQPGGSLRLSCAASGFTFSDYYMSWVRQAPGKGLEWVSGIYYDASWTYYADSVKGRFTISRDNSKNTLYLQMNSLRAEDTAVYYCAKGPLFCNDRTCSYYYAMDVWGQGTLVTVSS

SEQ ID NO: 106 - protein, 127 aa, Artificial Sequence
  Amino acid sequence of heavy chain variable region of affinity matured clone D12
EVQLLESGGGLVQPGGSLRLSCAASGFTFSDYYMSWVRQAPGKGLEWVSGIYYDASTKYYADSVKGRFTISRDNSKNTLYLQMNSLRAEDTAVYYCAKGPLFCNDRTCSYYYAMDVWGQGTLVTVSS

SEQ ID NO: 107 - protein, 127 aa, Artificial Sequence
  Amino acid sequence of heavy chain variable region of affinity matured clone E2
EVQLLESGGGLVQPGGSLRLSCAASGFTFSDYYMSWVRQAPGKGLEWVSGIYYDASIRYYADSVKGRFTISRDNSKNTLYLQMNSLRAEDTAVYYCAKGPLFCNDRTCSYYYAMDVWGQGTLVTVSS

SEQ ID NO: 108 - protein, 127 aa, Artificial Sequence
  Amino acid sequence of heavy chain variable region of affinity matured clone T2A1
EVQLLESGGGLVQPGGSLRLSCAASGFTFSDYYMSWVRQAPGKGLEWVSGIYYDASVKYYADSVKGRFTISRDNSKNTLYLQMNSLRAEDTAVYYCAKGPLFCNDRTCSYYYAMDVWGQGTLVTVSS

SEQ ID NO: 109 - protein, 127 aa, Artificial Sequence
  Amino acid sequence of heavy chain variable region of affinity matured clone T3H9
EVQLLESGGGLVQPGGSLRLSCAASGFTFSDYYMSWVRQAPGKGLEWVSGIYYDASAEYYADSVKGRFTISRDNSKNTLYLQMNSLRAEDTAVYYCAKGPLFCNDRTCSYYYAMDVWGQGTLVTVSS

SEQ ID NO: 110 - protein, 127 aa, Artificial Sequence
  Amino acid sequence of heavy chain variable region of affinity matured clone 2G1
EVQLLESGGGLVQPGGSLRLSCAASGFTFSDYYMSWVRQAPGKGLEWVSGIYYDSSTRYYADSVKGRFTISRDNSKNTLYLQMNSLRAEDTAVYYCAKGPLFCNDRTCSYYYAMDVWGQGTLVTVSS

SEQ ID NO: 111 - protein, 127 aa, Artificial Sequence
  Amino acid sequence of heavy chain variable region of affinity matured clone C4
EVQLLESGGGLVQPGGSLRLSCAASGFTFSDYYMSWVRQAPGKGLEWVSGIYYDSSMRYYADSVKGRFTISRDNSKNTLYLQMNSLRAEDTAVYYCAKGPLFCNDRTCSYYYAMDVWGQGTLVTVSS

SEQ ID NO: 112 - protein, 127 aa, Artificial Sequence; identical to SEQ ID NO: 111
  Amino acid sequence of heavy chain variable region of affinity matured clone C5

SEQ ID NO: 113 - protein, 127 aa, Artificial Sequence
  Amino acid sequence of heavy chain variable region of affinity matured clone D1
EVQLLESGGGLVQPGGSLRLSCAASGFTFSDYYMSWVRQAPGKGLEWVSGIYYDSSAKYYADSVKGRFTISRDNSKNTLYLQMNSLRAEDTAVYYCAKGPLFCNDRTCSYYYAMDVWGQGTLVTVSS

SEQ ID NO: 114 - protein, 127 aa, Artificial Sequence
  Amino acid sequence of heavy chain variable region of affinity matured clone D2
EVQLLESGGGLVQPGGSLRLSCAASGFTFSDYYMSWVRQAPGKGLEWVSGIYYDSSTDYYADSVKGRFTISRDNSKNTLYLQMNSLRAEDTAVYYCAKGPLFCNDRTCSYYYAMDVWGQGTLVTVSS

SEQ ID NO: 115 - protein, 127 aa, Artificial Sequence
  Amino acid sequence of heavy chain variable region of affinity matured clone E1
EVQLLESGGGLVQPGGSLRLSCAASGFTFSDYYMSWVRQAPGKGLEWVSGIYYDSSVTYYADSVKGRFTISRDNSKNTLYLQMNSLRAEDTAVYYCAKGPLFCNDRTCSYYYAMDVWGQGTLVTVSS

SEQ ID NO: 116 - protein, 127 aa, Artificial Sequence
  Amino acid sequence of heavy chain variable region of affinity matured clone F3
EVQLLESGGGLVQPGGSLRLSCAASGFTFSDYYMSWVRQAPGKGLEWVSGIYYDSSARYYADSVKGRFTISRDNSKNTLYLQMNSLRAEDTAVYYCAKGPLFCNDRTCSYYYAMDVWGQGTLVTVSS

SEQ ID NO: 117 - protein, 127 aa, Artificial Sequence
  Amino acid sequence of heavy chain variable region of affinity matured clone T2C1
EVQLLESGGGLVQPGGSLRLSCAASGFTFSDYYMSWVRQAPGKGLEWVSGIYYDSSQDYYADSVKGRFTISRDNSKNTLYLQMNSLRAEDTAVYYCAKGPLFCNDRTCSYYYAMDVWGQGTLVTVSS

SEQ ID NO: 118 - protein, 127 aa, Artificial Sequence; identical to SEQ ID NO: 117
  Amino acid sequence of heavy chain variable region of affinity matured clone T2H1

SEQ ID NO: 119 - protein, 127 aa, Artificial Sequence; identical to SEQ ID NO: 113
  Amino acid sequence of heavy chain variable region of affinity matured clone T2H5

SEQ ID NO: 120 - protein, 127 aa, Artificial Sequence
  Amino acid sequence of heavy chain variable region of affinity matured clone T3B8
EVQLLESGGGLVQPGGSLRLSCAASGFTFSDYYMSWVRQAPGKGLEWVSGIYYDSSVMYYADSVKGRFTISRDNSKNTLYLQMNSLRAEDTAVYYCAKGPLFCNDRTCSYYYAMDVWGQGTLVTVSS

SEQ ID NO: 121 - protein, 127 aa, Artificial Sequence
  Amino acid sequence of heavy chain variable region of affinity matured clone A12
EVQLLESGGGLVQPGGSLRLSCAASGFTFSDYYMSWVRQAPGKGLEWVSGIYYDGTVLYYADSVKGRFTISRDNSKNTLYLQMNSLRAEDTAVYYCAKGPLFCNDRTCSYYYAMDVWGQGTLVTVSS

SEQ ID NO: 122 - protein, 127 aa, Artificial Sequence
  Amino acid sequence of heavy chain variable region of affinity matured clone C2
EVQLLESGGGLVQPGGSLRLSCAASGFTFSDYYMSWVRQAPGKGLEWVSGIYYDGTNQYYADSVKGRFTISRDNSKNTLYLQMNSLRAEDTAVYYCAKGPLFCNDRTCSYYYAMDVWGQGTLVTVSS

SEQ ID NO: 123 - protein, 127 aa, Artificial Sequence
  Amino acid sequence of heavy chain variable region of affinity matured clone D7
EVQLLESGGGLVQPGGSLRLSCAASGFTFSDYYMSWVRQAPGKGLEWVSGIYYDGTAFYYADSVKGRFTISRDNSKNTLYLQMNSLRAEDTAVYYCAKGPLFCNDRTCSYYYAMDVWGQGTLVTVSS

SEQ ID NO: 124 - protein, 127 aa, Artificial Sequence
  Amino acid sequence of heavy chain variable region of affinity matured clone E3
EVQLLESGGGLVQPGGSLRLSCAASGFTFSDYYMSWVRQAPGKGLEWVSGIYYDGTAMYYADSVKGRFTISRDNSKNTLYLQMNSLRAEDTAVYYCAKGPLFCNDRTCSYYYAMDVWGQGTLVTVSS

SEQ ID NO: 125 - protein, 127 aa, Artificial Sequence
  Amino acid sequence of heavy chain variable region of affinity matured clone H10
EVQLLESGGGLVQPGGSLRLSCAASGFTFSDYYMSWVRQAPGKGLEWVSGIYYDGTNVYYADSVKGRFTISRDNSKNTLYLQMNSLRAEDTAVYYCAKGPLFCNDRTCSYYYAMDVWGQGTLVTVSS

SEQ ID NO: 126 - protein, 127 aa, Artificial Sequence
  Amino acid sequence of heavy chain variable region of affinity matured clone T3F5
EVQLLESGGGLVQPGGSLRLSCAASGFTFSDYYMSWVRQAPGKGLEWVSGIYYDGTAKYYADSVKGRFTISRDNSKNTLYLQMNSLRAEDTAVYYCAKGPLFCNDRTCSYYYAMDVWGQGTLVTVSS

SEQ ID NO: 127 - protein, 127 aa, Artificial Sequence
  Amino acid sequence of heavy chain variable region of affinity matured clone A10
EVQLLESGGGLVQPGGSLRLSCAASGFTFSDYYMSWVRQAPGKGLEWVSGIYYDGIYRYYADSVKGRFTISRDNSKNTLYLQMNSLRAEDTAVYYCAKGPLFCNDRTCSYYYAMDVWGQGTLVTVSS

SEQ ID NO: 128 - protein, 127 aa, Artificial Sequence
  Amino acid sequence of heavy chain variable region of affinity matured clone T3H1
EVQLLESGGGLVQPGGSLRLSCAASGFTFSDYYMSWVRQAPGKGLEWVSGIYYDGAVQYYADSVKGRFTISRDNSKNTLYLQMNSLRAEDTAVYYCAKGPLFCNDRTCSYYYAMDVWGQGTLVTVSS

SEQ ID NO: 129 - protein, 127 aa, Artificial Sequence
  Amino acid sequence of heavy chain variable region of affinity matured clone B1
EVQLLESGGGLVQPGGSLRLSCAASGFTFSDYYMSWVRQAPGKGLEWVSGIYYDGDVRYYADSVKGRFTISRDNSKNTLYLQMNSLRAEDTAVYYCAKGPLFCNDRTCSYYYAMDVWGQGTLVTVSS

SEQ ID NO: 130 - protein, 127 aa, Artificial Sequence
  Amino acid sequence of heavy chain variable region of affinity matured clone B7
EVQLLESGGGLVQPGGSLRLSCAASGFTFSDYYMSWVRQAPGKGLEWVSGIYYDGFAPYYADSVKGRFTISRDNSKNTLYLQMNSLRAEDTAVYYCAKGPLFCNDRTCSYYYAMDVWGQGTLVTVSS

SEQ ID NO: 131 - protein, 127 aa, Artificial Sequence
  Amino acid sequence of heavy chain variable region of affinity matured clone D8
EVQLLESGGGLVQPGGSLRLSCAASGFTFSDYYMSWVRQAPGKGLEWVSGIYYDGLHQYYADSVKGRFTISRDNSKNTLYLQMNSLRAEDTAVYYCAKGPLFCNDRTCSYYYAMDVWGQGTLVTVSS

SEQ ID NO: 132 - protein, 127 aa, Artificial Sequence
  Amino acid sequence of heavy chain variable region of affinity matured clone E12
EVQLLESGGGLVQPGGSLRLSCAASGFTFSDYYMSWVRQAPGKGLEWVSGIYYDSFVPYYADSVKGRFTISRDNSKNTLYLQMNSLRAEDTAVYYCAKGPLFCNDRTCSYYYAMDVWGQGTLVTVSS

SEQ ID NO: 133 - protein, 127 aa, Artificial Sequence
  Amino acid sequence of heavy chain variable region of affinity matured clone T2A12
EVQLLESGGGLVQPGGSLRLSCAASGFTFSDYYMSWVRQAPGKGLEWVSGIYYDGHQQYYADSVKGRFTISRDNSKNTLYLQMNSLRAEDTAVYYCAKGPLFCNDRTCSYYYAMDVWGQGTLVTVSS

SEQ ID NO: 134 - protein, 110 aa, Artificial Sequence
  Amino acid sequence of light chain variable region of CD19_8.1 antibody
QSVLTQPPSASGTPGQRVTISCTGSSSNIGSNAVYWYQQLPGTAPKLLIYDDNHRPSGVPDRFSGSKSGTSASLAISGLRSEDEADYYCGTWDYSLSGYVLGGGTKLTVL

SEQ ID NO: 135 - protein, 110 aa, Artificial Sequence
  Amino acid sequence of light chain variable region of affinity matured clone 2B1
QSVLTQPPSASGTPGQRVTISCVGGVSNIGSNAVYWYQQLPGTAPKLLIYDDNHRPSGVPDRFSGSKSGTSASLAISGLRSEDEADYYCGTWDYSLSGYVLGGGTKLTVL

SEQ ID NO: 136 - protein, 110 aa, Artificial Sequence
  Amino acid sequence of light chain variable region of affinity matured clone B12
QSVLTQPPSASGTPGQRVTISCAGHYSNIGSNAVYWYQQLPGTAPKLLIYDDNHRPSGVPDRFSGSKSGTSASLAISGLRSEDEADYYCGTWDYSLSGYVLGGGTKLTVL

SEQ ID NO: 137 - protein, 110 aa, Artificial Sequence
  Amino acid sequence of light chain variable region of affinity matured clone T2H3
QSVLTQPPSASGTPGQRVTISCGGGISNIGSNAVYWYQQLPGTAPKLLIYDDNHRPSGVPDRFSGSKSGTSASLAISGLRSEDEADYYCGTWDYSLSGYVLGGGTKLTVL

SEQ ID NO: 138 - protein, 110 aa, Artificial Sequence
  Amino acid sequence of light chain variable region of affinity matured clone T3C1
QSVLTQPPSASGTPGQRVTISCSGGPSNIGSNAVYWYQQLPGTAPKLLIYDDNHRPSGVPDRFSGSKSGTSASLAISGLRSEDEADYYCGTWDYSLSGYVLGGGTKLTVL

SEQ ID NO: 139 - protein, 110 aa, Artificial Sequence
  Amino acid sequence of light chain variable region of affinity matured clone D10
QSVLTQPPSASGTPGQRVTISCWGDYSNIGSNAVYWYQQLPGTAPKLLIYDDNHRPSGVPDRFSGSKSGTSASLAISGLRSEDEADYYCGTWDYSLSGYVLGGGTKLTVL

SEQ ID NO: 140 - protein, 110 aa, Artificial Sequence
  Amino acid sequence of light chain variable region of affinity matured clone F6
QSVLTQPPSASGTPGQRVTISCWGLPSNIGSNAVYWYQQLPGTAPKLLIYDDNHRPSGVPDRFSGSKSGTSASLAISGLRSEDEADYYCGTWDYSLSGYVLGGGTKLTVL

SEQ ID NO: 141 - protein, 110 aa, Artificial Sequence
  Amino acid sequence of light chain variable region of affinity matured clone B2
QSVLTQPPSASGTPGQRVTISCAGGVSNIGSNAVYWYQQLPGTAPKLLIYDDNHRPSGVPDRFSGSKSGTSASLAISGLRSEDEADYYCGTWDYSLSGYVLGGGTKLTVL

SEQ ID NO: 142 - protein, 110 aa, Artificial Sequence
  Amino acid sequence of light chain variable region of affinity matured clone B6
QSVLTQPPSASGTPGQRVTISCNGTPSNIGSNAVYWYQQLPGTAPKLLIYDDNHRPSGVPDRFSGSKSGTSASLAISGLRSEDEADYYCGTWDYSLSGYVLGGGTKLTVL

SEQ ID NO: 143 - protein, 110 aa, Artificial Sequence
  Amino acid sequence of light chain variable region of affinity matured clone 2F1
QSVLTQPPSASGTPGQRVTISCYGQPSNIGSNAVYWYQQLPGTAPKLLIYDDNHRPSGVPDRFSGSKSGTSASLAISGLRSEDEADYYCGTWDYSLSGYVLGGGTKLTVL

SEQ ID NO: 144 - protein, 110 aa, Artificial Sequence
  Amino acid sequence of light chain variable region of affinity matured clone C8
QSVLTQPPSASGTPGQRVTISCKGGMSNIGSNAVYWYQQLPGTAPKLLIYDDNHRPSGVPDRFSGSKSGTSASLAISGLRSEDEADYYCGTWDYSLSGYVLGGGTKLTVL

SEQ ID NO: 145 - protein, 110 aa, Artificial Sequence
  Amino acid sequence of light chain variable region of affinity matured clone D4
QSVLTQPPSASGTPGQRVTISCTGGVSNIGSNAVYWYQQLPGTAPKLLIYDDNHRPSGVPDRFSGSKSGTSASLAISGLRSEDEADYYCGTWDYSLSGYVLGGGTKLTVL

SEQ ID NO: 146 - protein, 110 aa, Artificial Sequence
  Amino acid sequence of light chain variable region of affinity matured clone B5
QSVLTQPPSASGTPGQRVTISCHGTPSNIGSNAVYWYQQLPGTAPKLLIYDDNHRPSGVPDRFSGSKSGTSASLAISGLRSEDEADYYCGTWDYSLSGYVLGGGTKLTVL

SEQ ID NO: 147 - protein, 110 aa, Artificial Sequence
  Amino acid sequence of light chain variable region of affinity matured clone G4
QSVLTQPPSASGTPGQRVTISCVGKPSNIGSNAVYWYQQLPGTAPKLLIYDDNHRPSGVPDRFSGSKSGTSASLAISGLRSEDEADYYCGTWDYSLSGYVLGGGTKLTVL

SEQ ID NO: 148 - protein, 110 aa, Artificial Sequence
  Amino acid sequence of light chain variable region of affinity matured clone A7
QSVLTQPPSASGTPGQRVTISCTGNPSNIGSNAVYWYQQLPGTAPKLLIYDDNHRPSGVPDRFSGSKSGTSASLAISGLRSEDEADYYCGTWDYSLSGYVLGGGTKLTVL

SEQ ID NO: 149 - protein, 110 aa, Artificial Sequence
  Amino acid sequence of light chain variable region of affinity matured clone D12
QSVLTQPPSASGTPGQRVTISCRGSASNIGSNAVYWYQQLPGTAPKLLIYDDNHRPSGVPDRFSGSKSGTSASLAISGLRSEDEADYYCGTWDYSLSGYVLGGGTKLTVL

SEQ ID NO: 150 - protein, 110 aa, Artificial Sequence
  Amino acid sequence of light chain variable region of affinity matured clone E2
QSVLTQPPSASGTPGQRVTISCKGMISNIGSNAVYWYQQLPGTAPKLLIYDDNHRPSGVPDRFSGSKSGTSASLAISGLRSEDEADYYCGTWDYSLSGYVLGGGTKLTVL

SEQ ID NO: 151 - protein, 110 aa, Artificial Sequence
  Amino acid sequence of light chain variable region of affinity matured clone T2A1
QSVLTQPPSASGTPGQRVTISCAGKPSNIGSNAVYWYQQLPGTAPKLLIYDDNHRPSGVPDRFSGSKSGTSASLAISGLRSEDEADYYCGTWDYSLSGYVLGGGTKLTVL

SEQ ID NO: 152 - protein, 110 aa, Artificial Sequence
  Amino acid sequence of light chain variable region of affinity matured clone T3H9
QSVLTQPPSASGTPGQRVTISCSGMLSNIGSNAVYWYQQLPGTAPKLLIYDDNHRPSGVPDRFSGSKSGTSASLAISGLRSEDEADYYCGTWDYSLSGYVLGGGTKLTVL

SEQ ID NO: 153 - protein, 110 aa, Artificial Sequence
  Amino acid sequence of light chain variable region of affinity matured clone 2G1
QSVLTQPPSASGTPGQRVTISCKGSFSNIGSNAVYWYQQLPGTAPKLLIYDDNHRPSGVPDRFSGSKSGTSASLAISGLRSEDEADYYCGTWDYSLSGYVLGGGTKLTVL

SEQ ID NO: 154 - protein, 110 aa, Artificial Sequence
  Amino acid sequence of light chain variable region of affinity matured clone C4
QSVLTQPPSASGTPGQRVTISCGGQPSNIGSNAVYWYQQLPGTAPKLLIYDDNHRPSGVPDRFSGSKSGTSASLAISGLRSEDEADYYCGTWDYSLSGYVLGGGTKLTVL

SEQ ID NO: 155 - protein, 110 aa, Artificial Sequence; identical to SEQ ID NO: 144
  Amino acid sequence of light chain variable region of affinity matured clone C5

SEQ ID NO: 156 - protein, 110 aa, Artificial Sequence; identical to SEQ ID NO: 138
  Amino acid sequence of light chain variable region of affinity matured clone D1

SEQ ID NO: 157 - protein, 110 aa, Artificial Sequence
  Amino acid sequence of light chain variable region of affinity matured clone D2
QSVLTQPPSASGTPGQRVTISCQGQPSNIGSNAVYWYQQLPGTAPKLLIYDDNHRPSGVPDRFSGSKSGTSASLAISGLRSEDEADYYCGTWDYSLSGYVLGGGTKLTVL

SEQ ID NO: 158 - protein, 110 aa, Artificial Sequence; identical to SEQ ID NO: 148
  Amino acid sequence of light chain variable region of affinity matured clone E1

SEQ ID NO: 159 - protein, 110 aa, Artificial Sequence
  Amino acid sequence of light chain variable region of affinity matured clone F3
QSVLTQPPSASGTPGQRVTISCTGSSSNIGSAPLYWYQQLPGTAPKLLIYDDNHRPSGVPDRFSGSKSGTSASLAISGLRSEDEADYYCGTWDYSLSGYVLGGGTKLTVL

SEQ ID NO: 160 - protein, 110 aa, Artificial Sequence
  Amino acid sequence of light chain variable region of affinity matured clone T2C1
QSVLTQPPSASGTPGQRVTISCRGGPSNIGSNAVYWYQQLPGTAPKLLIYDDNHRPSGVPDRFSGSKSGTSASLAISGLRSEDEADYYCGTWDYSLSGYVLGGGTKLTVL

SEQ ID NO: 161 - protein, 110 aa, Artificial Sequence
  Amino acid sequence of light chain variable region of affinity matured clone T2H1
QSVLTQPPSASGTPGQRVTISCQGGYSNIGSNAVYWYQQLPGTAPKLLIYDDNHRPSGVPDRFSGSKSGTSASLAISGLRSEDEADYYCGTWDYSLSGYVLGGGTKLTVL

SEQ ID NO: 162 - protein, 110 aa, Artificial Sequence
  Amino acid sequence of light chain variable region of affinity matured clone T2H5
QSVLTQPPSASGTPGQRVTISCSGNPSNIGSNAVYWYQQLPGTAPKLLIYDDNHRPSGVPDRFSGSKSGTSASLAISGLRSEDEADYYCGTWDYSLSGYVLGGGTKLTVL

SEQ ID NO: 163 - protein, 110 aa, Artificial Sequence
  Amino acid sequence of light chain variable region of affinity matured clone T3B8
QSVLTQPPSASGTPGQRVTISCEGSPSNIGSNAVYWYQQLPGTAPKLLIYDDNHRPSGVPDRFSGSKSGTSASLAISGLRSEDEADYYCGTWDYSLSGYVLGGGTKLTVL

SEQ ID NO: 164 - protein, 110 aa, Artificial Sequence
  Amino acid sequence of light chain variable region of affinity matured clone A12
QSVLTQPPSASGTPGQRVTISCQGGPSNIGSNAVYWYQQLPGTAPKLLIYDDNHRPSGVPDRFSGSKSGTSASLAISGLRSEDEADYYCGTWDYSLSGYVLGGGTKLTVL

SEQ ID NO: 165 - protein, 110 aa, Artificial Sequence
  Amino acid sequence of light chain variable region of affinity matured clone C2
QSVLTQPPSASGTPGQRVTISCTGGLSNIGSNAVYWYQQLPGTAPKLLIYDDNHRPSGVPDRFSGSKSGTSASLAISGLRSEDEADYYCGTWDYSLSGYVLGGGTKLTVL

SEQ ID NO: 166 - protein, 110 aa, Artificial Sequence
  Amino acid sequence of light chain variable region of affinity matured clone D7
QSVLTQPPSASGTPGQRVTISCEGQPSNIGSNAVYWYQQLPGTAPKLLIYDDNHRPSGVPDRFSGSKSGTSASLAISGLRSEDEADYYCGTWDYSLSGYVLGGGTKLTVL

SEQ ID NO: 167 - protein, 110 aa, Artificial Sequence
  Amino acid sequence of light chain variable region of affinity matured clone E3
QSVLTQPPSASGTPGQRVTISCSGGYSNIGSNAVYWYQQLPGTAPKLLIYDDNHRPSGVPDRFSGSKSGTSASLAISGLRSEDEADYYCGTWDYSLSGYVLGGGTKLTVL

SEQ ID NO: 168 - protein, 110 aa, Artificial Sequence
  Amino acid sequence of light chain variable region of affinity matured clone H10
QSVLTQPPSASGTPGQRVTISCLGGYSNIGSNAVYWYQQLPGTAPKLLIYDDNHRPSGVPDRFSGSKSGTSASLAISGLRSEDEADYYCGTWDYSLSGYVLGGGTKLTVL

SEQ ID NO: 169 - protein, 110 aa, Artificial Sequence
  Amino acid sequence of light chain variable region of affinity matured clone T3F5
QSVLTQPPSASGTPGQRVTISCHGQPSNIGSNAVYWYQQLPGTAPKLLIYDDNHRPSGVPDRFSGSKSGTSASLAISGLRSEDEADYYCGTWDYSLSGYVLGGGTKLTVL

SEQ ID NO: 170 - protein, 110 aa, Artificial Sequence
  Amino acid sequence of light chain variable region of affinity matured clone A10
QSVLTQPPSASGTPGQRVTISCSGDPSNIGSNAVYWYQQLPGTAPKLLIYDDNHRPSGVPDRFSGSKSGTSASLAISGLRSEDEADYYCGTWDYSLSGYVLGGGTKLTVL

SEQ ID NO: 171 - protein, 110 aa, Artificial Sequence
  Amino acid sequence of light chain variable region of affinity matured clone T3H1
QSVLTQPPSASGTPGQRVTISCDGGYSNIGSNAVYWYQQLPGTAPKLLIYDDNHRPSGVPDRFSGSKSGTSASLAISGLRSEDEADYYCGTWDYSLSGYVLGGGTKLTVL

SEQ ID NO: 172 - protein, 110 aa, Artificial Sequence
  Amino acid sequence of light chain variable region of affinity matured clone B1
QSVLTQPPSASGTPGQRVTISCVGSPSNIGSNAVYWYQQLPGTAPKLLIYDDNHRPSGVPDRFSGSKSGTSASLAISGLRSEDEADYYCGTWDYSLSGYVLGGGTKLTVL

SEQ ID NO: 173 - protein, 110 aa, Artificial Sequence
  Amino acid sequence of light chain variable region of affinity matured clone B7
QSVLTQPPSASGTPGQRVTISCRGTPSNIGSNAVYWYQQLPGTAPKLLIYDDNHRPSGVPDRFSGSKSGTSASLAISGLRSEDEADYYCGTWDYSLSGYVLGGGTKLTVL

SEQ ID NO: 174 - protein, 110 aa, Artificial Sequence
  Amino acid sequence of light chain variable region of affinity matured clone D8
QSVLTQPPSASGTPGQRVTISCVGNLSNIGSNAVYWYQQLPGTAPKLLIYDDNHRPSGVPDRFSGSKSGTSASLAISGLRSEDEADYYCGTWDYSLSGYVLGGGTKLTVL

SEQ ID NO: 175 - protein, 110 aa, Artificial Sequence
  Amino acid sequence of light chain variable region of affinity matured clone E12
QSVLTQPPSASGTPGQRVTISCAGSASNIGSNAVYWYQQLPGTAPKLLIYDDNHRPSGVPDRFSGSKSGTSASLAISGLRSEDEADYYCGTWDYSLSGYVLGGGTKLTVL

SEQ ID NO: 176 - protein, 110 aa, Artificial Sequence
  Amino acid sequence of light chain variable region of affinity matured clone T2A12
QSVLTQPPSASGTPGQRVTISCTGSSSNIGSAPTYWYQQLPGTAPKLLIYDDNHRPSGVPDRFSGSKSGTSASLAISGLRSEDEADYYCGTWDYSLSGYVLGGGTKLTVL

SEQ ID NO: 177 - DNA, 60 bp, Artificial Sequence
  Nucleotide sequence for encoding CD8 leader
atggccctgcctgtgaccgctctgctgctgcccctggctctgctgctgcacgccgctcgc

SEQ ID NO: 178 - DNA, 207 bp, Artificial Sequence
  Nucleotide sequence for encoding CD8 hinge/transmembrain domain
accacaactccagctccccggccccctacccctgcaccaacaatcgccagccagcctctgtccctgagaccagaggcatgtaggccagctgcaggaggagcagtgcatacaagaggcctggacttcgcctgcgatatctacatttgggctcctctggcaggaacttgtggcgtgctgctgctgtctctggtcatcaccctgtactgc

SEQ ID NO: 179 - DNA, 126 bp, Artificial Sequence
  Nucleotide sequence for encoding intracellular domain of CD137
aaaaggggccgcaagaaactgctgtatattttcaagcagcccttcatgcggcccgtgcagaccacacaggaggaagacgggtgctcctgtagattccccgaggaagaggaaggcgggtgtgagctg

SEQ ID NO: 180 - DNA, 336 bp, Artificial Sequence
  Nucleotide sequence for encoding intracellular domain of CD3-zeta
cgcgtcaagttcagccgatcagccgatgctcctgcatacaagcagggccagaatcagctgtataacgagctgaatctggggcgccgagaggaatacgacgtgctggataagcggagagggagggaccccgaaatgggaggcaaacctaggcgcaagaacccacaggagggactgtacaatgaactgcagaaggacaaaatggccgaggcttattccgaaattgggatgaaaggagagcgacggagagggaagggacacgatgggctgtatcagggactgtctaccgccactaaagatacctacgacgctctgcacatgcaggctctgccacctcgc

SEQ ID NO: 181 - DNA, 1518 bp, Artificial Sequence
  Nucleotide sequence of CAR construct comprising CD19_8.1 scFv
atggccctgcctgtgaccgctctgctgctgcccctggctctgctgctgcacgccgctcgccccgtggcccaggcggccgaggtgcagctgttggagtctgggggaggcttggtacagcctggggggtccctgagactctcctgtgcagcctctggattcacctttagcgattattatatgagctgggtccgccaggctccagggaaggggctggagtgggtctcagggatctattatgatgatagtagtcaatattacgctgattctgtaaaaggtcggttcaccatctccagagacaattccaagaacacgctgtatctgcaaatgaacagcctgagagccgaggacacggccgtgtattactgtgcgaaaggtcctcttttttgtaatgatcggacttgttcttattattatgctatggacgtctggggccagggtacactggtcaccgtgagctcaggtggaggcggttcaggcggaggtggatccggcggtggcggatcgcagtctgtgctgactcagccaccctcagcgtctgggacccccgggcagagggtcaccatctcttgtactggctcttcatctaatattggcagtaatgctgtctactggtaccagcagctaccaggaacggcccccaaactcctcatctatgatgataatcatcggccaagcggggtccctgaccgattctctggctccaagtctggcacctcagcctccctggccatcagtgggctccggtccgaggatgaggctgattattactgtggtacctgggattatagcctgagtggttatgtcttaggcggaggcaccaagctgacggtcctaggccaggccggccagaccacaactccagctccccggccccctacccctgcaccaacaatcgccagccagcctctgtccctgagaccagaggcatgtaggccagctgcaggaggagcagtgcatacaagaggcctggacttcgcctgcgatatctacatttgggctcctctggcaggaacttgtggcgtgctgctgctgtctctggtcatcaccctgtactgcaaaaggggccgcaagaaactgctgtatattttcaagcagcccttcatgcggcccgtgcagaccacacaggaggaagacgggtgctcctgtagattccccgaggaagaggaaggcgggtgtgagctgcgcgtcaagttcagccgatcagccgatgctcctgcatacaagcagggccagaatcagctgtataacgagctgaatctggggcgccgagaggaatacgacgtgctggataagcggagagggagggaccccgaaatgggaggcaaacctaggcgcaagaacccacaggagggactgtacaatgaactgcagaaggacaaaatggccgaggcttattccgaaattgggatgaaaggagagcgacggagagggaagggacacgatgggctgtatcagggactgtctaccgccactaaagatacctacgacgctctgcacatgcaggctctgccacctcgc

SEQ ID NO: 182 - DNA, 15 bp, Artificial Sequence
  Nucleotide sequence for encoding CDRH1 of CD19_8.1 antibody
gattattatatgagc

SEQ ID NO: 183 - DNA, 51 bp, Artificial Sequence
  Nucleotide sequence for encoding CDRH2 of CD19_8.1 antibody
gggatctattatgatgatagtagtcaatattacgctgattctgtaaaaggt

SEQ ID NO: 184 - DNA, 54 bp, Artificial Sequence
  Nucleotide sequence for encoding CDRH3 of CD19_8.1 antibody
ggtcctcttttttgtaatgatcggacttgttcttattattatgctatggacgtc

SEQ ID NO: 185 - DNA, 39 bp, Artificial Sequence
  Nucleotide sequence for encoding CDRL1 of CD19_8.1 antibody
actggctcttcatctaatattggcagtaatgctgtctac

SEQ ID NO: 186 - DNA, 21 bp, Artificial Sequence
  Nucleotide sequence for encoding CDRL2 of CD19_8.1 antibody
gatgataatcatcggccaagc

SEQ ID NO: 187 - DNA, 33 bp, Artificial Sequence
  Nucleotide sequence for encoding CDRL3 of CD19_8.1 antibody
ggtacctgggattatagcctgagtggttatgtc

SEQ ID NO: 188 - DNA, 381 bp, Artificial Sequence
  Nucleotide sequence for encoding heavy chain variable region of CD19_8.1 antibody
gaggtgcagctgttggagtctgggggaggcttggtacagcctggggggtccctgagactctcctgtgcagcctctggattcacctttagcgattattatatgagctgggtccgccaggctccagggaaggggctggagtgggtctcagggatctattatgatgatagtagtcaatattacgctgattctgtaaaaggtcggttcaccatctccagagacaattccaagaacacgctgtatctgcaaatgaacagcctgagagccgaggacacggccgtgtattactgtgcgaaaggtcctcttttttgtaatgatcggacttgttcttattattatgctatggacgtctggggccagggtacactggtcaccgtgagctca

SEQ ID NO: 189 - DNA, 330 bp, Artificial Sequence
  Nucleotide sequence for encoding light chain variable region of CD19_8.1 antibody
cagtctgtgctgactcagccaccctcagcgtctgggacccccgggcagagggtcaccatctcttgtactggctcttcatctaatattggcagtaatgctgtctactggtaccagcagctaccaggaacggcccccaaactcctcatctatgatgataatcatcggccaagcggggtccctgaccgattctctggctccaagtctggcacctcagcctccctggccatcagtgggctccggtccgaggatgaggctgattattactgtggtacctgggattatagcctgagtggttatgtcttaggcggaggcaccaagctgacggtccta

SEQ ID NO: 190 - protein, 17 aa, Artificial Sequence
  CDRH2 of CD19_8.1_3C12, 6F10, 7D2, 7H11, 8E8, 10D3, 10E5, 10H4
GIYYDGSAKYYADSVKG

SEQ ID NO: 191 - protein, 18 aa, Artificial Sequence
  CDRH3 of CD19_8.1_3C12
GPNFCNDRTCSYYYAMDV

SEQ ID NO: 192 - protein, 18 aa, Artificial Sequence
  CDRH3 of CD19_8.1_6F10
GPLFCNDRTCSYYYAMDV

SEQ ID NO: 193 - protein, 18 aa, Artificial Sequence
  CDRH3 of CD19_8.1_7D2
GPLFCNDNTCSYYYAMDV

SEQ ID NO: 194 - protein, 18 aa, Artificial Sequence
  CDRH3 of CD19_8.1_7H11
GPLFCNDDTCSYYYAMDV

SEQ ID NO: 195 - protein, 18 aa, Artificial Sequence
  CDRH3 of CD19_8.1_8E8
GPLFCNDRDCSYYYAMDV

SEQ ID NO: 196 - protein, 18 aa, Artificial Sequence
  CDRH3 of CD19_8.1_10D3
GPLFCNDRTCSMYYAMDV

SEQ ID NO: 197 - protein, 18 aa, Artificial Sequence
  CDRH3 of CD19_8.1_10E5
GPLFCNDRTCSMYYAMDV

SEQ ID NO: 198 - protein, 18 aa, Artificial Sequence
  CDRH3 of CD19_8.1_10H4
GPLFCNDRTCSKYYAMDV

SEQ ID NO: 199 - protein, 13 aa, Artificial Sequence
  CDRL1 of CD19_8.1_3C12, 6F10, 7D2, 7H11, 8E8, 10E5, 10H4
YGQPSNIGSNAVY

SEQ ID NO: 200 - protein, 13 aa, Artificial Sequence
  CDRL1 of CD19_8.1_10D3
TGGPSNIGSNAVY